European Patent Application EP 4 324 923 A1, published February 21, 2024. Title: RNA Inhibitor for Inhibiting Hepatitis B Virus Gene Expression and Application Thereof. Applicant: KYLONOVA (XIAMEN) BIOPHARMA CO., LTD. The sequence listing filed with the application follows.

SEQUENCE LISTING (4 sequences)

SEQ ID NO: 1 - RNA, 19 nt, Artificial Sequence
  Sense strand
ggguuuuucucguugacaa

SEQ ID NO: 2 - RNA, 21 nt, Artificial Sequence
  Antisense strand
uugucaacgagaaaaacccuu

SEQ ID NO: 3 - RNA, 19 nt, Artificial Sequence
  Sense strand
ggguuuuucuuguugacaa

SEQ ID NO: 4 - RNA, 21 nt, Artificial Sequence
  Antisense strand
uugucaacaagaaaaacccuu